European Patent Application EP 4 534 564 A1, published April 9, 2025. Title: RECOMBINANT FUSION PROTEIN TARGETING PD-L1 AND VEGF AND PREPARATION AND USES THEREOF. Applicant: ImmuneOnco Biopharmaceuticals (Shanghai) Inc. Application EP EP23815201.1, filed May 30, 2023. The sequence listing filed with the application follows.

SEQUENCE LISTING (27 sequences)

SEQ ID NO: 1 - protein, 8 aa, synthetic construct
GYTFTSNW

SEQ ID NO: 2 - protein, 8 aa, synthetic construct
IHPNSGSS

SEQ ID NO: 3 - protein, 14 aa, synthetic construct
ARSYYGSSPYYFDY

SEQ ID NO: 4 - protein, 6 aa, synthetic construct
QDIINY

SEQ ID NO: 5 - protein, 9 aa, synthetic construct
QQGDTLPWT

SEQ ID NO: 6 - protein, 344 aa, synthetic construct
MGWSCIILFLVATATGVHSSDTGRPFVEMYSEIPEIIHMTEGRELVIPCRVTSPNITVTLKKFPLDTLIPDGKRIIWDSRKGFIISNATYKEIGLLTCEATVNGHLYKTNYLTHRQTNTTTTPAPRPPTPAPTIASQPLSLRPEACRPAAGGAVHTRGLDFACDFWVLVVVGGVLACYSLLVTVAFIIFWVRSKRSRLLHSDYMNMTPRRPGPTRKHYQPYAPPRDFAAYRSRVKFSRSAEPPAYQQGQNQLYNELNLGRREEYDVLDKRRGRDPEMGGKPRRKNPQEGLYNELQKDKMAEAYSEIGMKGERRRGKGHDGLYQGLSTATKDTYDALHMQALPPR

SEQ ID NO: 7 - protein, 121 aa, synthetic construct
QVQLVQSGAEVKKPGASVKVSCKASGYTFTSNWMHWVRQAPGQGLEWMGMIHPNSGSSNYNEKFKSRVTMTRDTSTSTVYMELSSLRSEDTAVYYCARSYYGSSPYYFDYWGQGTLVTVSS

SEQ ID NO: 8 - protein, 107 aa, synthetic construct
DIQMTQSPSSLSASVGDRVTITCRASQDIINYLNWYQQKPGKAPKLLIYYTSRLHSGVPSRFSGSGSGTDFTFTISSLQPEDIATYYCQQGDTLPWTFGQGTKVEIK

SEQ ID NO: 9 - protein, 330 aa, synthetic construct
ASTKGPSVFPLAPSSKSTSGGTAALGCLVKDYFPEPVTVSWNSGALTSGVHTFPAVLQSSGLYSLSSVVTVPSSSLGTQTYICNVNHKPSNTKVDKRVEPKSCDKTHTCPPCPAPELLGGPSVFLFPPKPKDTLMISRTPEVTCVVVDVSHEDPEVKFNWYVDGVEVHNAKTKPREEQYNATYRVVSVLTVLHQDWLNGKEYKCKVSNKALPAPIAATISKAKGQPREPQVYTLPPSREEMTKNQVSLTCLVKGFYPSDIAVEWESNGQPENNYKTTPPVLDSDGSFFLYSKLTVDKSRWQQGNVFSCSVMHEALHNHYTQKSLSLSPGK

SEQ ID NO: 10 - protein, 107 aa, synthetic construct [sequence omitted]

SEQ ID NO: 11 - protein, 100 aa, Homo sapiens
SDTGRPFVEMYSEIPEIIHMTEGRELVIPCRVTSPNITVTLKKFPLDTLIPDGKRIIWDSRKGFIISAATYKEIGLLTCEATVNGHLYKTNYLTHRQTNT

SEQ ID NO: 12 - protein, 15 aa, synthetic construct
GGGGSGGGGSGGGGS

SEQ ID NO: 13 - protein, 566 aa, synthetic construct
SDTGRPFVEMYSEIPEIIHMTEGRELVIPCRVTSPNITVTLKKFPLDTLIPDGKRIIWDSRKGFIISAATYKEIGLLTCEATVNGHLYKTNYLTHRQTNTGGGGSGGGGSGGGGSQVQLVQSGAEVKKPGASVKVSCKASGYTFTSNWMHWVRQAPGQGLEWMGMIHPNSGSSNYNEKFKSRVTMTRDTSTSTVYMELSSLRSEDTAVYYCARSYYGSSPYYFDYWGQGTLVTVSSASTKGPSVFPLAPSSKSTSGGTAALGCLVKDYFPEPVTVSWNSGALTSGVHTFPAVLQSSGLYSLSSVVTVPSSSLGTQTYICNVNHKPSNTKVDKRVEPKSCDKTHTCPPCPAPELLGGPSVFLFPPKPKDTLMISRTPEVTCVVVDVSHEDPEVKFNWYVDGVEVHNAKTKPREEQYNATYRVVSVLTVLHQDWLNGKEYKCKVSNKALPAPIAATISKAKGQPREPQVYTLPPSREEMTKNQVSLTCLVKGFYPSDIAVEWESNGQPENNYKTTPPVLDSDGSFFLYSKLTVDKSRWQQGNVFSCSVMHEALHNHYTQKSLSLSPGK

SEQ ID NO: 14 - protein, 214 aa, synthetic construct
DIQMTQSPSSLSASVGDRVTITCRASQDIINYLNWYQQKPGKAPKLLIYYTSRLHSGVPSRFSGSGSGTDFTFTISSLQPEDIATYYCQQGDTLPWTFGQGTKVEIKRTVAAPSVFIFPPSDEQLKSGTASVVCLLNNFYPREAKVQWKVDNALQSGNSQESVTEQDSKDSTYSLSSTLTLSKADYEKHKVYACEVTHQGLSSPVTKSFNRGEC

SEQ ID NO: 15 - protein, 451 aa, synthetic construct
QVQLVQSGAEVKKPGASVKVSCKASGYTFTSNWMHWVRQAPGQGLEWMGMIHPNSGSSNYNEKFKSRVTMTRDTSTSTVYMELSSLRSEDTAVYYCARSYYGSSPYYFDYWGQGTLVTVSSASTKGPSVFPLAPSSKSTSGGTAALGCLVKDYFPEPVTVSWNSGALTSGVHTFPAVLQSSGLYSLSSVVTVPSSSLGTQTYICNVNHKPSNTKVDKRVEPKSCDKTHTCPPCPAPELLGGPSVFLFPPKPKDTLMISRTPEVTCVVVDVSHEDPEVKFNWYVDGVEVHNAKTKPREEQYNATYRVVSVLTVLHQDWLNGKEYKCKVSNKALPAPIAATISKAKGQPREPQVYTLPPSREEMTKNQVSLTCLVKGFYPSDIAVEWESNGQPENNYKTTPPVLDSDGSFFLYSKLTVDKSRWQQGNVFSCSVMHEALHNHYTQKSLSLSPGK

SEQ ID NO: 16 - protein, 329 aa, synthetic construct
SDTGRPFVEMYSEIPEIIHMTEGRELVIPCRVTSPNITVTLKKFPLDTLIPDGKRIIWDSRKGFIISAATYKEIGLLTCEATVNGHLYKTNYLTHRQTNTGGGGSGGGGSGGGGSDIQMTQSPSSLSASVGDRVTITCRASQDIINYLNWYQQKPGKAPKLLIYYTSRLHSGVPSRFSGSGSGTDFTFTISSLQPEDIATYYCQQGDTLPWTFGQGTKVEIKRTVAAPSVFIFPPSDEQLKSGTASVVCLLNNFYPREAKVQWKVDNALQSGNSQESVTEQDSKDSTYSLSSTLTLSKADYEKHKVYACEVTHQGLSSPVTKSFNRGEC

SEQ ID NO: 17 - protein, 563 aa, synthetic construct
SDTGRPFVEMYSEIPEIIHMTEGRELVIPCRVTSPNITVTLKKFPLDTLIPDGKRIIWDSRKGFIISAATYKEIGLLTCEATVNGHLYKTNYLTHRQTNTGGGGSGGGGSGGGGSEVQLVESGGGLVQPGGSLRLSCAASGFTFSDSWIHWVRQAPGKGLEWVAWISPYGGSTYYADSVKGRFTISADTSKNTAYLQMNSLRAEDTAVYYCARRHWPGGFDYWGQGTLVTVSSASTKGPSVFPLAPSSKSTSGGTAALGCLVKDYFPEPVTVSWNSGALTSGVHTFPAVLQSSGLYSLSSVVTVPSSSLGTQTYICNVNHKPSNTKVDKRVEPKSCDKTHTCPPCPAPELLGGPSVFLFPPKPKDTLMISRTPEVTCVVVDVSHEDPEVKFNWYVDGVEVHNAKTKPREEQYNATYRVVSVLTVLHQDWLNGKEYKCKVSNKALPAPIAATISKAKGQPREPQVYTLPPSREEMTKNQVSLTCLVKGFYPSDIAVEWESNGQPENNYKTTPPVLDSDGSFFLYSKLTVDKSRWQQGNVFSCSVMHEALHNHYTQKSLSLSPGK

SEQ ID NO: 18 - protein, 214 aa, synthetic construct
DIQMTQSPSSLSASVGDRVTITCRASQDVSTAVAWYQQKPGKAPKLLIYSASFLYSGVPSRFSGSGSGTDFTLTISSLQPEDFATYYCQQYLYHPATFGQGTKVEIKRTVAAPSVFIFPPSDEQLKSGTASVVCLLNNFYPREAKVQWKVDNALQSGNSQESVTEQDSKDSTYSLSSTLTLSKADYEKHKVYACEVTHQGLSSPVTKSFNRGEC

SEQ ID NO: 19 - protein, 334 aa, synthetic construct
SDTGRPFVEMYSEIPEIIHMTEGRELVIPCRVTSPNITVTLKKFPLDTLIPDGKRIIWDSRKGFIISAATYKEIGLLTCEATVNGHLYKTNYLTHRQTNTEFEPKSCDKTHTCPPCPAPELLGGPSVFLFPPKPKDTLMISRTPEVTCVVVDVSHEDPEVKFNWYVDGVEVHNAKTKPREEQYNSTYRVVSVLTVLHQDWLNGKEYKCKVSNKALPAPIEKTISKAKGQPREPQVYTLPPSRDELTKNQVSLTCLVKGFYPSDIAVEWESNGQPENNYKTTPPVLDSDGSFFLYSKLTVDKSRWQQGNVFSCSVMHEALHNHYTQKSLSLSPGK

SEQ ID NO: 20 - protein, 232 aa, synthetic construct
EPKSCDKTHTCPPCPAPELLGGPSVFLFPPKPKDTLMISRTPEVTCVVVDVSHEDPEVKFNWYVDGVEVHNAKTKPREEQYNSTYRVVSVLTVLHQDWLNGKEYKCKVSNKALPAPIEKTISKAKGQPREPQVYTLPPSRDELTKNQVSLTCLVKGFYPSDIAVEWESNGQPENNYKTTPPVLDSDGSFFLYSKLTVDKSRWQQGNVFSCSVMHEALHNHYTQKSLSLSPGK

SEQ ID NO: 21 - DNA, 57 bp, synthetic construct
  source 1..57: mol_type = other DNA
atgggatggtcatgtatcatcctttttctggtagcaactgcaactggagtacattca

SEQ ID NO: 22 - protein, 391 aa, synthetic construct
MGWSCIILFLVATATGVHSLDSPDRPWNPPTFSPALLVVTEGDAATFTCSFSNTSESFVLNWYRMSPSNQTDKLAAFPEDRSQPGQDCRFRVTQLPNGRDFHMSVVRARRNDSGTYLCGAISLAPKAQIKESLRAELRVTERRAEVPTAHPSPSPRPAGQFQEFVPRDCGCKPCICTVPEVSSVFIFPPKPKDVLTITLTPKVTCVVVDISKDDPEVQFSWFVDDVEVHTAQTQPREEQFNSTFRSVSELPIMHQDWLNGKEFKCRVNSAAFPAPIEKTISKTKGRPKAPQVYTIPPPKEQMAKDKVSLTCMITDFFPEDITVEWQWNGQPAENYKNTQPIMNTNGSYFVYSKLNVQKSNWEAGNTFTCSVLHEGLHNHHTEKSLSHSPGK

SEQ ID NO: 23 - DNA, 1758 bp, synthetic construct
  source 1..1758: mol_type = other DNA
atgggatggtcatgtatcatcctttttctggtagcaactgcaactggagtacattcaagtgatacaggtagacctttcgtagagatgtacagtgaaatccccgaaattatacacatgactgaaggaagggagctcgtcattccctgccgggttacgtcacctaacatcactgttactttaaaaaagtttccacttgacactttgatccctgatggaaaacgcataatctgggacagtagaaagggcttcatcatatcagctgcaacgtacaaagaaatagggcttctgacctgtgaagcaacagtcaatgggcatttgtataagacaaactatctcacacatcgacaaaccaatacaggcggcggtgggagcggcggcggtgggagcggcggcgggggctcgcaagtgcagctggtgcagagcggcgccgaggtgaagaagcctggcgcaagcgtgaaggtgagctgcaaggcaagcggctacaccttcacaagcaactggatgcactgggtgagacaagcccctggccaaggcctggagtggatgggcatgatccaccctaacagcggcagcagcaactacaacgagaagttcaagagcagagtgaccatgacaagagacacaagcacaagcaccgtgtacatggagctgagcagcctgagaagcgaggacaccgccgtgtactactgcgctagaagctactacggcagcagcccttactacttcgactactggggccaaggcaccctggtgaccgtgagcagcgctagcaccaagggcccatcggtcttccccctggcaccctcctccaagagcacctctgggggcacagcggccctgggctgcctggtcaaggactacttccccgaaccggtgacggtgtcgtggaactcaggcgccctgaccagcggcgtgcacaccttcccggctgtcctacagtcctcaggactctactccctcagcagcgtggtgaccgtgccctccagcagcttgggcacccagacctacatctgcaacgtgaatcacaagcccagcaacaccaaggtggacaagagagttgagcccaaatcttgtgacaaaactcacacatgcccaccgtgcccagcacctgaactcctggggggaccgtcagtcttcctcttccccccaaaacccaaggacaccctcatgatctcccggacccctgaggtcacatgcgtggtggtggacgtgagccacgaagaccctgaggtcaagttcaactggtatgtggacggcgtggaggtgcataatgccaagacaaagccgcgggaggagcagtacaacgccacgtaccgtgtggtcagcgtcctcaccgtcctgcaccaagactggctgaatggcaaggagtacaagtgcaaggtctccaacaaagccctcccagcccccatcgccgcaaccatctccaaagccaaagggcagccccgagaaccacaggtgtacaccctgcccccatcccgggaggagatgaccaagaaccaagtcagcctgacctgcctggtcaaaggcttctatcccagcgacatcgccgtggagtgggagagcaatgggcagccggagaacaactacaagaccacgcctcccgtgctggactccgacggctccttcttcctctattccaagctcaccgtggacaagagcaggtggcagcaggggaacgtcttctcatgctccgtgatgcatgaggctctgcacaaccactacacgcagaagagcctctccctgtctccgggcaaatga

SEQ ID NO: 24 - DNA, 841 bp, synthetic construct
  source 1..841: mol_type = other DNA
atgggatggtcatgtatcatcctttttctggtagcaactgcaactggagtacattcagacattcagatgacacagagccctagcagcctgagcgcaagcgtgggcgacagagtgaccatcacctgcagagcaagccaagacatcatcaactacctgaactggtatcagcagaagcctggcaaggcccctaagctgctgatctactacacaagcagactgcacagcggcgtgcctagcagattcagcggcagcggcagcggcaccgacttcaccttcaccatcagcagcctgcagcctgaggacatcgccacctactactgtcagcaaggcgacaccctgccttggaccttcggccaaggcaccaaggtggagatcaagcgtgagttctagaggatccatctgggataagcatgctgttttctgtctgtccctaacatgccctgtgattatccgcaaacaacacacccaagggcagaactttgttacttaaacaccatcctgtttgcttctttcctcaggaactgtggctgcaccatctgtcttcatcttcccgccatctgatgagcagttgaaatctggaactgcctctgttgtgtgcctgctgaataacttctatcccagagaggccaaagtacagtggaaggtggataacgccctccaatcgggtaactcccaggagagtgtcacagagcaggacagcaaggacagcacctacagcctcagcagcaccctgacgctgagcaaagcagactacgagaaacacaaagtctacgcctgcgaagtcacccatcagggcctgagctcgcccgtcacaaagagcttcaacaggggagagtgttag

SEQ ID NO: 25 - DNA, 1413 bp, synthetic construct
  source 1..1413: mol_type = other DNA
atgggatggtcatgtatcatcctttttctggtagcaactgcaactggagtacattcacaagtgcagctggtgcagagcggcgccgaggtgaagaagcctggcgcaagcgtgaaggtgagctgcaaggcaagcggctacaccttcacaagcaactggatgcactgggtgagacaagcccctggccaaggcctggagtggatgggcatgatccaccctaacagcggcagcagcaactacaacgagaagttcaagagcagagtgaccatgacaagagacacaagcacaagcaccgtgtacatggagctgagcagcctgagaagcgaggacaccgccgtgtactactgcgctagaagctactacggcagcagcccttactacttcgactactggggccaaggcaccctggtgaccgtgagcagcgctagcaccaagggcccatcggtcttccccctggcaccctcctccaagagcacctctgggggcacagcggccctgggctgcctggtcaaggactacttccccgaaccggtgacggtgtcgtggaactcaggcgccctgaccagcggcgtgcacaccttcccggctgtcctacagtcctcaggactctactccctcagcagcgtggtgaccgtgccctccagcagcttgggcacccagacctacatctgcaacgtgaatcacaagcccagcaacaccaaggtggacaagagagttgagcccaaatcttgtgacaaaactcacacatgcccaccgtgcccagcacctgaactcctggggggaccgtcagtcttcctcttccccccaaaacccaaggacaccctcatgatctcccggacccctgaggtcacatgcgtggtggtggacgtgagccacgaagaccctgaggtcaagttcaactggtatgtggacggcgtggaggtgcataatgccaagacaaagccgcgggaggagcagtacaacgccacgtaccgtgtggtcagcgtcctcaccgtcctgcaccaagactggctgaatggcaaggagtacaagtgcaaggtctccaacaaagccctcccagcccccatcgccgcaaccatctccaaagccaaagggcagccccgagaaccacaggtgtacaccctgcccccatcccgggaggagatgaccaagaaccaagtcagcctgacctgcctggtcaaaggcttctatcccagcgacatcgccgtggagtgggagagcaatgggcagccggagaacaactacaagaccacgcctcccgtgctggactccgacggctccttcttcctctattccaagctcaccgtggacaagagcaggtggcagcaggggaacgtcttctcatgctccgtgatgcatgaggctctgcacaaccactacacgcagaagagcctctccctgtctccgggcaaatga

SEQ ID NO: 26 - DNA, 1186 bp, synthetic construct
  source 1..1186: mol_type = other DNA
atgggatggtcatgtatcatcctttttctggtagcaactgcaactggagtacattcaagtgatacaggtagacctttcgtagagatgtacagtgaaatccccgaaattatacacatgactgaaggaagggagctcgtcattccctgccgggttacgtcacctaacatcactgttactttaaaaaagtttccacttgacactttgatccctgatggaaaacgcataatctgggacagtagaaagggcttcatcatatcagctgcaacgtacaaagaaatagggcttctgacctgtgaagcaacagtcaatgggcatttgtataagacaaactatctcacacatcgacaaaccaatacaggcggcggtgggagcggcggcggtgggagcggcggcgggggctcggacattcagatgacacagagccctagcagcctgagcgcaagcgtgggcgacagagtgaccatcacctgcagagcaagccaagacatcatcaactacctgaactggtatcagcagaagcctggcaaggcccctaagctgctgatctactacacaagcagactgcacagcggcgtgcctagcagattcagcggcagcggcagcggcaccgacttcaccttcaccatcagcagcctgcagcctgaggacatcgccacctactactgtcagcaaggcgacaccctgccttggaccttcggccaaggcaccaaggtggagatcaagcgtgagttctagaggatccatctgggataagcatgctgttttctgtctgtccctaacatgccctgtgattatccgcaaacaacacacccaagggcagaactttgttacttaaacaccatcctgtttgcttctttcctcaggaactgtggctgcaccatctgtcttcatcttcccgccatctgatgagcagttgaaatctggaactgcctctgttgtgtgcctgctgaataacttctatcccagagaggccaaagtacagtggaaggtggataacgccctccaatcgggtaactcccaggagagtgtcacagagcaggacagcaaggacagcacctacagcctcagcagcaccctgacgctgagcaaagcagactacgagaaacacaaagtctacgcctgcgaagtcacccatcagggcctgagctcgcccgtcacaaagagcttcaacaggggagagtgttag

SEQ ID NO: 27 - protein, 418 aa, synthetic construct
MGWSCIILFLVATATGVHSAPMAEGGGQNHHEVVKFMDVYQRSYCHPIETLVDIFQEYPDEIEYIFKPSCVPLMRCGGCCNDEGLECVPTEESNITMQIMRIKPHQGQHIGEMSFLQHNKCECRPKKDRARQENPCGPCSERRKHLFVQDPQTCKCSCKNTDSRCKARQLELNERTCRCDKPRREFEPKSCDKTHTCPPCPAPELLGGPSVFLFPPKPKDTLMISRTPEVTCVVVDVSHEDPEVKFNWYVDGVEVHNAKTKPREEQYNSTYRVVSVLTVLHQDWLNGKEYKCKVSNKALPAPIEKTISKAKGQPREPQVYTLPPSRDELTKNQVSLTCLVKGFYPSDIAVEWESNGQPENNYKTTPPVLDSDGSFFLYSKLTVDKSRWQQGNVFSCSVMHEALHNHYTQKSLSLSPGK